European Patent Application EP 4 768 126 A2, published July 1, 2026. Title: SYSTEMS, METHODS, AND APPARATUS FOR AUTOMATED SELF-CONTAINED BIOLOGICAL ANALYSIS. Applicant: Co-Diagnostics, Inc. Application WO PCT/US2022/027476, filed May 3, 2022. The sequence listing filed with the application follows.

SEQUENCE LISTING (5 sequences)

SEQ ID NO: 1 - DNA, 26 bp, synthetic construct
  misc_feature 1..26: note = PCR primer
  source 1..26: mol_type = other DNA
cgaggtagtgtattattagtgggaag

SEQ ID NO: 2 - DNA, 21 bp, synthetic construct
  misc_feature 1..21: note = PCR primer
  source 1..21: mol_type = other DNA
agggagatgatgtagcactca

SEQ ID NO: 3 - DNA, 49 bp, synthetic construct
  misc_feature 1..49: note = oligonucleotide
  source 1..49: mol_type = other DNA
cggaatcttgcacgccctcgctcaggccttcgtcactggtcccgccacc

SEQ ID NO: 4 - DNA, 19 bp, synthetic construct
  misc_feature 1..19: note = oligonucleotide
  source 1..19: mol_type = other DNA
agtggaacctcatcaggaa

SEQ ID NO: 5 - DNA, 25 bp, synthetic construct
  misc_feature 1..25: note = oligonucleotide
  source 1..25: mol_type = other DNA
ctcctgatgaggttccacctggttt